European Patent Specification EP 3 224 352 B1, published January 3, 2024. Title: Reprogramming-based models of neurodevelopmental disorders and uses thereof. Applicant: IEO IRCCS Casa Sollievo della Sofferenza Universita' degli Studi di Milano Testa, Giuseppe Atashpazgargari, Sina Adamo, Antonio Germain, Pierre-Luc Merla , Giuseppe D'Agostino, Giuseppe Zanella, Matteo. The sequence listing filed with the application follows.

SEQUENCE LISTING (32 sequences)

SEQ ID NO: 1 - DNA, 20 bp, Artificial Sequence
  synthetic primer
gcaccgtcaaggctgagaac

SEQ ID NO: 2 - DNA, 19 bp, Artificial Sequence
  synthetic primer
agggatctcgctcctggaa

SEQ ID NO: 3 - DNA, 21 bp, Artificial Sequence
  synthetic primer
ggaaaaggaaaaggtcagtgc

SEQ ID NO: 4 - DNA, 21 bp, Artificial Sequence
  synthetic primer
gtttatctgctcttccgaggg

SEQ ID NO: 5 - DNA, 21 bp, Artificial Sequence
  synthetic primer
gatcttgcaaccctgaaatgg

SEQ ID NO: 6 - DNA, 23 bp, Artificial Sequence
  synthetic primer
cacctggagatagtattgacctg

SEQ ID NO: 7 - DNA, 21 bp, Artificial Sequence
  synthetic primer
gctgccatcttcctctggtaa

SEQ ID NO: 8 - DNA, 21 bp, Artificial Sequence
  synthetic primer
gctgccatcttcctctggtaa

SEQ ID NO: 9 - DNA, 22 bp, Artificial Sequence
  synthetic primer
cctcctgcatagcttcaacaaa

SEQ ID NO: 10 - DNA, 19 bp, Artificial Sequence
  synthetic primer
ggtcagagggcaacacaga

SEQ ID NO: 11 - DNA, 19 bp, Artificial Sequence
  synthetic primer
caccagcccttgacatcag

SEQ ID NO: 12 - DNA, 22 bp, Artificial Sequence
  synthetic primer
tccctccaactctaccctttag

SEQ ID NO: 13 - DNA, 21 bp, Artificial Sequence
  synthetic primer
tgatgtggagagtttgagtgg

SEQ ID NO: 14 - DNA, 21 bp, Artificial Sequence
  synthetic primer
gaaaagatgaggaagggacgg

SEQ ID NO: 15 - DNA, 20 bp, Artificial Sequence
  synthetic primer
atgttaagggagcagtgagc

SEQ ID NO: 16 - DNA, 21 bp, Artificial Sequence
  synthetic primer
atggtcagctctcaagaatgg

SEQ ID NO: 17 - DNA, 21 bp, Artificial Sequence
  synthetic primer
gaacccagatctcttacgctg

SEQ ID NO: 18 - DNA, 22 bp, Artificial Sequence
  synthetic primer
catctttaatcccctgcctctc

SEQ ID NO: 19 - DNA, 21 bp, Artificial Sequence
  synthetic primer
ggaaaccagattagagacggg

SEQ ID NO: 20 - DNA, 22 bp, Artificial Sequence
  synthetic primer
gtttgtagttacctctccagcg

SEQ ID NO: 21 - DNA, 21 bp, Artificial Sequence
  synthetic primer
gaaatcaagcctcccaaagtg

SEQ ID NO: 22 - DNA, 19 bp, Artificial Sequence
  synthetic primer
tggagaggcagaaggaaaa

SEQ ID NO: 23 - DNA, 21 bp, Artificial Sequence
  synthetic primer
aagccttctccggtcataatg

SEQ ID NO: 24 - DNA, 20 bp, Artificial Sequence
  synthetic primer
tgatgtccgtgtttctcagg

SEQ ID NO: 25 - DNA, 20 bp, Artificial Sequence
  synthetic primer
cctgtgaactgaggttcctg

SEQ ID NO: 26 - DNA, 21 bp, Artificial Sequence
  synthetic primer
ccactgaagactcctgctaag

SEQ ID NO: 27 - DNA, 19 bp, Artificial Sequence
  synthetic primer
acaagcccgaagtccaaag

SEQ ID NO: 28 - DNA, 18 bp, Artificial Sequence
  synthetic primer
tcctgttcctgcacaacg

SEQ ID NO: 29 - DNA, 20 bp, Artificial Sequence
  synthetic primer
cctcaaccagaaacaagcag

SEQ ID NO: 30 - DNA, 21 bp, Artificial Sequence
  synthetic primer
ccaccgaccctttagctttag

SEQ ID NO: 31 - DNA, 21 bp, Artificial Sequence
  synthetic primer
gctcctgtaattagtgtcggg

SEQ ID NO: 32 - DNA, 21 bp, Artificial Sequence
  synthetic primer
gggatcacttttcagggtcag